European Patent Specification EP 3 532 497 B1, published July 24, 2024. Title: MODIFIED IMMUNOGLOBULIN HINGE REGIONS TO REDUCE. Applicant: THE BOARD OF TRUSTEES OF THE LELAND STANFORD JUNIOR UNIVERSITY. The sequence listing filed with the application follows.

SEQUENCE LISTING (8 sequences)

SEQ ID NO: 1 - protein, 98 aa, Homo sapiens
ASTKGPSVFPLAPCSRSTSESTAALGCLVKDYFPEPVTVSWNSGALTSGVHTFPAVLQSSGLYSLSSVVTVPSSSLGTKTYTCNVDHKPSNTKVDKRV

SEQ ID NO: 2 - protein, 12 aa, Homo sapiens
ESKYGPPCPSCP

SEQ ID NO: 3 - protein, 110 aa, Homo sapiens
APEFLGGPSVFLFPPKPKDTLMISRTPEVTCVVVDVSQEDPEVQFNWYVDGVEVHNAKTKPREEQFNSTYRVVSVLTVLHQDWLNGKEYKCKVSNKGLPSSIEKTISKAK

SEQ ID NO: 4 - protein, 107 aa, Homo sapiens
GQPREPQVYTLPPSQEEMTKNQVSLTCLVKGFYPSDIAVEWESNGQPENNYKTTPPVLDSDGSFFLYSRLTVDKSRWQEGNVFSCSVMHEALHNHYTQKSLSLSLGK

SEQ ID NO: 5 - protein, 7 aa, Artificial Sequence
  Synthetic Sequence
  Misc_feature (5)..(5): X is S or P
PPCPXCP

SEQ ID NO: 6 - protein, 439 aa, Artificial Sequence
  Synthetic Sequence
QVQLVQSGAEVKKPGASVKVSCKASGYTFTNYNMHWVRQAPGQRLEWMGTIYPGNDDTSYNQKFKDRVTITADTSASTAYMELSSLRSEDTAVYYCARGGYRAMDYWGQGTLVTVSSASTKGPSVFPLAPCSRSTSESTAALGCLVKDYFPEPVTVSWNSGALTSGVHTFPAVLQSSGLYSLSSVVTVPSSSLGTKTYTCNVDHKPSNTKVDKRVPPCPPCPAPEFLGGPSVFLFPPKPKDTLMISRTPEVTCVVVDVSQEDPEVQFNWYVDGVEVHNAKTKPREEQFNSTYRVVSVLTVLHQDWLNGKEYKCKVSNKGLPSSIEKTISKAKGQPREPQVYTLPPSQEEMTKNQVSLTCLVKGFYPSDIAVEWESNGQPENNYKTTPPVLDSDGSFFLYSRLTVDKSRWQEGNVFSCSVMHEALHNHYTQKSLSLSLGK

SEQ ID NO: 7 - protein, 434 aa, Artificial Sequence
  Synthetic Sequence
DVVMTQSPLSLPVTPGEPASISCRSSQSIVYSNGNTYLGWYLQKPGQSPKLLIYKVSNRFSGVPDRFSGSGSGTDFTLKISRVEAEDVGVYHCFQGSHVPYTFGGGTKVEIKASTKGPSVFPLAPCSRSTSESTAALGCLVKDYFPEPVTVSWNSGALTSGVHTFPAVLQSSGLYSLSSVVTVPSSSLGTKTYTCNVDHKPSNTKVDKRVPPCPPCPAPEFLGGPSVFLFPPKPKDTLMISRTPEVTCVVVDVSQEDPEVQFNWYVDGVEVHNAKTKPREEQFNSTYRVVSVLTVLHQDWLNGKEYKCKVSNKGLPSSIEKTISKAKGQPREPQVYTLPPSQEEMTKNQVSLTCLVKGFYPSDIAVEWESNGQPENNYKTTPPVLDSDGSFFLYSRLTVDKSRWQEGNVFSCSVMHEALHNHYTQKSLSLSLGK

SEQ ID NO: 8 - protein, 12 aa, Artificial Sequence
  Synthetic Sequence
  Misc_feature (10)..(10): X is S or P
ESKYGPPCPXCP